European Patent Specification EP 3 283 521 B1, published November 15, 2023. Title: DRUG CONJUGATES COMPRISING ANTIBODIES AGAINST CLAUDIN 18.2. Applicant: Ganymed Pharmaceuticals AG. The sequence listing filed with the application follows.

SEQUENCE LISTING (51 sequences)

SEQ ID NO: 1 - protein, 261 aa, Homo sapiens
MAVTACQGLGFVVSLIGIAGIIAATCMDQWSTQDLYNNPVTAVFNYQGLWRSCVRESSGFTECRGYFTLLGLPAMLQAVRALMIVGIVLGAIGLLVSIFALKCIRIGSMEDSAKANMTLTSGIMFIVSGLCAIAGVSVFANMLVTNFWMSTANMYTGMGGMVQTVQTRYTFGAALFVGWVAGGLTLIGGVMMCIACRGLAPEETNYKAVSYHASGHSVAYKPGGFKASTGFGSNTKNKKIYDGGARTEDEVQSYPSKHDYV

SEQ ID NO: 2 - protein, 261 aa, Homo sapiens
MSTTTCQVVAFLLSILGLAGCIAATGMDMWSTQDLYDNPVTSVFQYEGLWRSCVRQSSGFTECRPYFTILGLPAMLQAVRALMIVGIVLGAIGLLVSIFALKCIRIGSMEDSAKANMTLTSGIMFIVSGLCAIAGVSVFANMLVTNFWMSTANMYTGMGGMVQTVQTRYTFGAALFVGWVAGGLTLIGGVMMCIACRGLAPEETNYKAVSYHASGHSVAYKPGGFKASTGFGSNTKNKKIYDGGARTEDEVQSYPSKHDYV

SEQ ID NO: 3 - protein, 10 aa, Homo sapiens
DQWSTQDLYN

SEQ ID NO: 4 - protein, 11 aa, Homo sapiens
NNPVTAVFNYQ

SEQ ID NO: 5 - protein, 14 aa, Homo sapiens
STQDLYNNPVTAVF

SEQ ID NO: 6 - protein, 13 aa, Homo sapiens
TNFWMSTANMYTG

SEQ ID NO: 7 - protein, 13 aa, Homo sapiens
DSAKANMTLTSGI

SEQ ID NO: 8 - protein, 55 aa, Homo sapiens
MDQWSTQDLYNNPVTAVFNYQGLWRSCVRESSGFTECRGYFTLLGLPAMLQAVRA

SEQ ID NO: 9 - protein, 24 aa, Homo sapiens
FALKCIRIGSMEDSAKANMTLTSG

SEQ ID NO: 10 - protein, 40 aa, Homo sapiens
ANMLVTNFWMSTANMYTGMGGMVQTVQTRYTFGAALFVGW

SEQ ID NO: 11 - protein, 153 aa, Homo sapiens
MDQWSTQDLYNNPVTAVFNYQGLWRSCVRESSGFTECRGYFTLLGLPAMLQAVRALMIVGIVLGAIGLLVSIFALKCIRIGSMEDSAKANMTLTSGIMFIVSGLCAIAGVSVFANMLVTNFWMSTANMYTGMGGMVQTVQTRYTFGAALFVGW

SEQ ID NO: 12 - protein, 107 aa, Artificial [sequence omitted]

SEQ ID NO: 13 - protein, 326 aa, Artificial
  Description of artificial sequence: Translation of PCR product
GPSVFPLAPSSKSTSGGTAALGCLVKDYFPEPVTVSWNSGALTSGVHTFPAVLQSSGLYSLSSVVTVPSSSLGTQTYICNVNHKPSNTKVDKKVEPKSCDKTHTCPPCPAPELLGGPSVFLFPPKPKDTLMISRTPEVTCVVVDVSHEDPEVKFNWYVDGVEVHNAKTKPREEQYNSTYRVVSVLTVLHQDWLNGKEYKCKVSNKALPAPIEKTISKAKGQPREPQVYTLPPSRDELTKNQVSLTCLVKGFYPSDIAVEWESNGQPENNYKTTPPVLDSDGSFFLYSKLTVDKSRWQQGNVFSCSVMHEALHNHYTQKSLSLSPGK

SEQ ID NO: 14 - protein, 466 aa, Artificial
  Description of artificial sequence: chimeric monoclonal antibody
MEWTWVFLFLLSVTAGVHSQVQLQQSGAELMKPGASVKISCKATGYTFSSYWIEWVKQRPGHGLEWIGEILPGSGSTNYNEKFKGKATFTADTSSNTAYMQLSSLTSEDSAVYYCARYDYPWFAYWGQGTLVTVSAASTKGPSVFPLAPSSKSTSGGTAALGCLVKDYFPEPVTVSWNSGALTSGVHTFPAVLQSSGLYSLSSVVTVPSSSLGTQTYICNVNHKPSNTKVDKKVEPKSCDKTHTCPPCPAPELLGGPSVFLFPPKPKDTLMISRTPEVTCVVVDVSHEDPEVKFNWYVDGVEVHNAKTKPREEQYNSTYRVVSVLTVLHQDWLNGKEYKCKVSNKALPAPIEKTISKAKGQPREPQVYTLPPSRDELTKNQVSLTCLVKGFYPSDIAVEWESNGQPENNYKTTPPVLDSDGSFFLYSKLTVDKSRWQQGNVFSCSVMHEALHNHYTQKSLSLSPGK

SEQ ID NO: 15 - protein, 467 aa, Artificial
  Description of artificial sequence: chimeric monoclonal antibody
MDWLWNLLFLMAAAQSIQAQIQLVQSGPELKKPGETVKISCKASGYTFTNYGMNWVKQAPGKGLKWMGWINTNTGEPTYAEEFKGRFAFSLETSASTAYLQINNLKNEDTATYFCARLGFGNAMDYWGQGTSVTVSSASTKGPSVFPLAPSSKSTSGGTAALGCLVKDYFPEPVTVSWNSGALTSGVHTFPAVLQSSGLYSLSSVVTVPSSSLGTQTYICNVNHKPSNTKVDKKVEPKSCDKTHTCPPCPAPELLGGPSVFLFPPKPKDTLMISRTPEVTCVVVDVSHEDPEVKFNWYVDGVEVHNAKTKPREEQYNSTYRVVSVLTVLHQDWLNGKEYKCKVSNKALPAPIEKTISKAKGQPREPQVYTLPPSRDELTKNQVSLTCLVKGFYPSDIAVEWESNGQPENNYKTTPPVLDSDGSFFLYSKLTVDKSRWQQGNVFSCSVMHEALHNHYTQKSLSLSPGK

SEQ ID NO: 16 - protein, 465 aa, Artificial
  Description of artificial sequence: chimeric monoclonal antibody
MEWIWIFLFILSGTAGVHSQVQLQQSGAELARPGASVKLSCKASGYTFTDYYINWVKQRTGQGLEWIGEIYPGSGNTYYNEKFKGKATLTADKSSSTAYMQLSSLTSEDSAVYFCARSYGAFDYWGQGTTLTVSSASTKGPSVFPLAPSSKSTSGGTAALGCLVKDYFPEPVTVSWNSGALTSGVHTFPAVLQSSGLYSLSSVVTVPSSSLGTQTYICNVNHKPSNTKVDKKVEPKSCDKTHTCPPCPAPELLGGPSVFLFPPKPKDTLMISRTPEVTCVVVDVSHEDPEVKFNWYVDGVEVHNAKTKPREEQYNSTYRVVSVLTVLHQDWLNGKEYKCKVSNKALPAPIEKTISKAKGQPREPQVYTLPPSRDELTKNQVSLTCLVKGFYPSDIAVEWESNGQPENNYKTTPPVLDSDGSFFLYSKLTVDKSRWQQGNVFSCSVMHEALHNHYTQKSLSLSPGK

SEQ ID NO: 17 - protein, 467 aa, Artificial
  Description of artificial sequence: chimeric monoclonal antibody
MGWSCIILFLVATATGVHSQVQLQQPGAELVRPGASVKLSCKASGYTFTSYWINWVKQRPGQGLEWIGNIYPSDSYTNYNQKFKDKATLTVDKSSSTAYMQLSSPTSEDSAVYYCTRSWRGNSFDYWGQGTTLTVSSASTKGPSVFPLAPSSKSTSGGTAALGCLVKDYFPEPVTVSWNSGALTSGVHTFPAVLQSSGLYSLSSVVTVPSSSLGTQTYICNVNHKPSNTKVDKKVEPKSCDKTHTCPPCPAPELLGGPSVFLFPPKPKDTLMISRTPEVTCVVVDVSHEDPEVKFNWYVDGVEVHNAKTKPREEQYNSTYRVVSVLTVLHQDWLNGKEYKCKVSNKALPAPIEKTISKAKGQPREPQVYTLPPSRDELTKNQVSLTCLVKGFYPSDIAVEWESNGQPENNYKTTPPVLDSDGSFFLYSKLTVDKSRWQQGNVFSCSVMHEALHNHYTQKSLSLSPGK

SEQ ID NO: 18 - protein, 466 aa, Artificial
  Description of artificial sequence: chimeric monoclonal antibody
MEWRIFLFILSGTAGVHSQVQLQQSGPELVKPGASVKMSCKASGYTFTDYVISWVKQRTGQGLEWIGEIYPGSGSTYYNEKFKGKATLTADKSSNTAYMQLSSLTSEDSAVYFCARGVLLRAMDYWGQGTSVTVSSASTKGPSVFPLAPSSKSTSGGTAALGCLVKDYFPEPVTVSWNSGALTSGVHTFPAVLQSSGLYSLSSVVTVPSSSLGTQTYICNVNHKPSNTKVDKKVEPKSCDKTHTCPPCPAPELLGGPSVFLFPPKPKDTLMISRTPEVTCVVVDVSHEDPEVKFNWYVDGVEVHNAKTKPREEQYNSTYRVVSVLTVLHQDWLNGKEYKCKVSNKALPAPIEKTISKAKGQPREPQVYTLPPSRDELTKNQVSLTCLVKGFYPSDIAVEWESNGQPENNYKTTPPVLDSDGSFFLYSKLTVDKSRWQQGNVFSCSVMHEALHNHYTQKSLSLSPGK

SEQ ID NO: 19 - protein, 469 aa, Artificial [sequence omitted]

SEQ ID NO: 20 - protein, 240 aa, Artificial
  Description of artificial sequence: chimeric monoclonal antibody
MESQTQVLMSLLFWVSGTCGDIVMTQSPSSLTVTAGEKVTMSCKSSQSLLNSGNQKNYLTWYQQKPGQPPKLLIYWASTRESGVPDRFTGSGSGTDFTLTISSVQAEDLAVYYCQNDYSYPLTFGAGTKLELKRTVAAPSVFIFPPSDEQLKSGTASVVCLLNNFYPREAKVQWKVDNALQSGNSQESVTEQDSKDSTYSLSSTLTLSKADYEKHKVYACEVTHQGLSSPVTKSFNRGEC

SEQ ID NO: 21 - protein, 235 aa, Artificial
  Description of artificial sequence: chimeric monoclonal antibody
MHFQVQIFSFLLISASVIMSRGQIVLTQSPAIMSASPGEKVTITCSASSSVSYMHWFQQKPGTSPKLWIYSTSNLASGVPARFSGSGSGTSYSLTISRMEAEDAATYYCQQRSSYPPTFGGGTKLEIKRTVAAPSVFIFPPSDEQLKSGTASVVCLLNNFYPREAKVQWKVDNALQSGNSQESVTEQDSKDSTYSLSSTLTLSKADYEKHKVYACEVTHQGLSSPVTKSFNRGEC

SEQ ID NO: 22 - protein, 234 aa, Artificial
  Description of artificial sequence: chimeric monoclonal antibody
MEFQTQVFVFVLLWLSGVDGDIVMTQSQKFMSTSVGDRVSITCKASQNVRTAVAWYQQKPGQSPKALIYLASNRHTGVPDRFTGSGSGTDFTLTISNVQSEDLADYFCLQHWNYPLTFGGGTKLEIKRTVAAPSVFIFPPSDEQLKSGTASVVCLLNNFYPREAKVQWKVDNALQSGNSQESVTEQDSKDSTYSLSSTLTLSKADYEKHKVYACEVTHQGLSSPVTKSFNRGEC

SEQ ID NO: 23 - protein, 240 aa, Artificial
  Description of artificial sequence: chimeric monoclonal antibody
MDSQAQVLMLLLLWVSGTCGDIVMSQSPSSLAVSVGEKVTMSCKSSQSLLYSSNQKNYLAWYQQKPGQSPKLLIYWASTRESGVPDRFTGSGSGTDFTLTISSVKAEDLAVYYCQQYYSYPLTFGAGTKLELKRTVAAPSVFIFPPSDEQLKSGTASVVCLLNNFYPREAKVQWKVDNALQSGNSQESVTEQDSKDSTYSLSSTLTLSKADYEKHKVYACEVTHQGLSSPVTKSFNRGEC

SEQ ID NO: 24 - protein, 240 aa, Artificial
  Description of artificial sequence: chimeric monoclonal antibody
MESQTQVLMSLLFWVSGTCGDIVMTQSPSSLTVTAGEKVTMSCKSSQSLLNSGNQKNYLTWYQQKPGQPPKLLIYWASTRESGVPDRFTGSGSGTDFTLTISSVQAEDLAVYYCQNDYSYPFTFGSGTKLEIKRTVAAPSVFIFPPSDEQLKSGTASVVCLLNNFYPREAKVQWKVDNALQSGNSQESVTEQDSKDSTYSLSSTLTLSKADYEKHKVYACEVTHQGLSSPVTKSFNRGEC

SEQ ID NO: 25 - protein, 239 aa, Artificial
  Description of artificial sequence: chimeric monoclonal antibody
MDSQAQVLILLLLWVSGTCGDIVMSQSPSSLAVSAGEKVTMSCKSSQSLLNSRTRKNYLAWYQQKPGQSPKLLIYWASTRESGVPDRFTGSGSGTDFTLTISSVQAEDLAVYYCKQSYNLYTFGGGTKLEIKRTVAAPSVFIFPPSDEQLKSGTASVVCLLNNFYPREAKVQWKVDNALQSGNSQESVTEQDSKDSTYSLSSTLTLSKADYEKHKVYACEVTHQGLSSPVTKSFNRGEC

SEQ ID NO: 26 - protein, 240 aa, Artificial
  Description of artificial sequence: chimeric monoclonal antibody
MDSQAQVLMLLLLWVSGTCGDIVMSQSPSSLAVSVGEKVTMSCKSSQSLLYSSNQKNYLAWYQQKPGQSPKLLIYWASTRESGVPDRFTGSGSATDFTLTISSVQAEDLADYHCGQGYSYPYTFGGGTKLEIKRTVAAPSVFIFPPSDEQLKSGTASVVCLLNNFYPREAKVQWKVDNALQSGNSQESVTEQDSKDSTYSLSSTLTLSKADYEKHKVYACEVTHQGLSSPVTKSFNRGEC

SEQ ID NO: 27 - protein, 240 aa, Artificial; identical to SEQ ID NO: 23
  Description of artificial sequence: chimeric monoclonal antibody

SEQ ID NO: 28 - protein, 234 aa, Artificial
  Description of artificial sequence: chimeric monoclonal antibody
MESQTLVFISILLWLYGADGNIVMTQSPKSMSMSVGERVTLTCKASENVVTYVSWYQQKPEQSPKLLIYGASNRYTGVPDRFTGSGSATDFTLTISSVKAEDLAVYYCQQYYSYPLTFGAGTKLELKRTVAAPSVFIFPPSDEQLKSGTASVVCLLNNFYPREAKVQWKVDNALQSGNSQESVTEQDSKDSTYSLSSTLTLSKADYEKHKVYACEVTHQGLSSPVTKSFNRGEC

SEQ ID NO: 29 - protein, 117 aa, Artificial
  Description of artificial sequence: Translation of PCR product
QVQLQQSGAELMKPGASVKISCKATGYTFSSYWIEWVKQRPGHGLEWIGEILPGSGSTNYNEKFKGKATFTADTSSNTAYMQLSSLTSEDSAVYYCARYDYPWFAYWGQGTLVTVSA

SEQ ID NO: 30 - protein, 118 aa, Artificial
  Description of artificial sequence: Translation of PCR product
QIQLVQSGPELKKPGETVKISCKASGYTFTNYGMNWVKQAPGKGLKWMGWINTNTGEPTYAEEFKGRFAFSLETSASTAYLQINNLKNEDTATYFCARLGFGNAMDYWGQGTSVTVSS

SEQ ID NO: 31 - protein, 116 aa, Artificial
  Description of artificial sequence: Translation of PCR product
QVQLQQSGAELARPGASVKLSCKASGYTFTDYYINWVKQRTGQGLEWIGEIYPGSGNTYYNEKFKGKATLTADKSSSTAYMQLSSLTSEDSAVYFCARSYGAFDYWGQGTTLTVSS

SEQ ID NO: 32 - protein, 118 aa, Artificial
  Description of artificial sequence: Translation of PCR product
QVQLQQPGAELVRPGASVKLSCKASGYTFTSYWINWVKQRPGQGLEWIGNIYPSDSYTNYNQKFKDKATLTVDKSSSTAYMQLSSPTSEDSAVYYCTRSWRGNSFDYWGQGTTLTVSS

SEQ ID NO: 33 - protein, 118 aa, Artificial
  Description of artificial sequence: Translation of PCR product
QVQLQQSGPELVKPGASVKMSCKASGYTFTDYVISWVKQRTGQGLEWIGEIYPGSGSTYYNEKFKGKATLTADKSSNTAYMQLSSLTSEDSAVYFCARGVLLRAMDYWGQGTSVTVSS

SEQ ID NO: 34 - protein, 120 aa, Artificial
  Description of artificial sequence: Translation of PCR product
QVHLQQSGSELRSPGSSVKLSCKDFDSEVFPFAYMSWIRQKPGHGFEWIGDILPSIGRTIYGEKFEDKATLDADTVSNTAYLELNSLTSEDSAIYYCARGEGYGAWFAYWGQGTLVTVSA

SEQ ID NO: 35 - protein, 113 aa, Artificial
  Description of artificial sequence: Translation of PCR product
DIVMTQSPSSLTVTAGEKVTMSCKSSQSLLNSGNQKNYLTWYQQKPGQPPKLLIYWASTRESGVPDRFTGSGSGTDFTLTISSVQAEDLAVYYCQNDYSYPLTFGAGTKLELK

SEQ ID NO: 36 - protein, 106 aa, Artificial
  Description of artificial sequence: Translation of PCR product
QIVLTQSPAIMSASPGEKVTITCSASSSVSYMHWFQQKPGTSPKLWIYSTSNLASGVPARFSGSGSGTSYSLTISRMEAEDAATYYCQQRSSYPPTFGGGTKLEIK

SEQ ID NO: 37 - protein, 107 aa, Artificial
  Description of artificial sequence: Translation of PCR product
DIVMTQSQKFMSTSVGDRVSITCKASQNVRTAVAWYQQKPGQSPKALIYLASNRHTGVPDRFTGSGSGTDFTLTISNVQSEDLADYFCLQHWNYPLTFGGGTKLEIK

SEQ ID NO: 38 - protein, 113 aa, Artificial
  Description of artificial sequence: Translation of PCR product
DIVMSQSPSSLAVSVGEKVTMSCKSSQSLLYSSNQKNYLAWYQQKPGQSPKLLIYWASTRESGVPDRFTGSGSGTDFTLTISSVKAEDLAVYYCQQYYSYPLTFGAGTKLELK

SEQ ID NO: 39 - protein, 113 aa, Artificial
  Description of artificial sequence: Translation of PCR product
DIVMTQSPSSLTVTAGEKVTMSCKSSQSLLNSGNQKNYLTWYQQKPGQPPKLLIYWASTRESGVPDRFTGSGSGTDFTLTISSVQAEDLAVYYCQNDYSYPFTFGSGTKLEIK

SEQ ID NO: 40 - protein, 112 aa, Artificial
  Description of artificial sequence: Translation of PCR product
DIVMSQSPSSLAVSAGEKVTMSCKSSQSLLNSRTRKNYLAWYQQKPGQSPKLLIYWASTRESGVPDRFTGSGSGTDFTLTISSVQAEDLAVYYCKQSYNLYTFGGGTKLEIK

SEQ ID NO: 41 - protein, 113 aa, Artificial
  Description of artificial sequence: Translation of PCR product
DIVMSQSPSSLAVSVGEKVTMSCKSSQSLLYSSNQKNYLAWYQQKPGQSPKLLIYWASTRESGVPDRFTGSGSATDFTLTISSVQAEDLADYHCGQGYSYPYTFGGGTKLEIK

SEQ ID NO: 42 - protein, 113 aa, Artificial; identical to SEQ ID NO: 38
  Description of artificial sequence: Translation of PCR product

SEQ ID NO: 43 - protein, 107 aa, Artificial
  Description of artificial sequence: Translation of PCR product
NIVMTQSPKSMSMSVGERVTLTCKASENVVTYVSWYQQKPEQSPKLLIYGASNRYTGVPDRFTGSGSATDFTLTISSVKAEDLAVYYCQQYYSYPLTFGAGTKLELK

SEQ ID NO: 44 - protein, 15 aa, Artificial
  Epitope
MDQWSTQDLYNNPVT

SEQ ID NO: 45 - protein, 15 aa, Artificial
  Epitope
STQDLYNNPVTAVFN

SEQ ID NO: 46 - protein, 15 aa, Artificial
  Epitope
LYNNPVTAVFNYQGL

SEQ ID NO: 47 - protein, 15 aa, Artificial
  Epitope
PVTAVFNYQGLWRSC

SEQ ID NO: 48 - protein, 15 aa, Artificial
  Epitope
VFNYQGLWRSCVRES

SEQ ID NO: 49 - protein, 15 aa, Artificial
  Epitope
QGLWRSCVRESSGFT

SEQ ID NO: 50 - protein, 15 aa, Artificial
  Epitope
RSCVRESSGFTECRG

SEQ ID NO: 51 - protein, 467 aa, Artificial Sequence
  chimeric monoclonal antibody
MGWSCIILFLVATATGVHSQVQLQQPGAELVRPGASVKLSCKASGYTFTSYWINWVKQRPGQGLEWIGNIYPSDSYTNYNQKFKDKATLTVDKSSSTAYMQLSSPTSEDSAVYYCTRSWRGNSFDYWGQGTTLTVSSASTKGPSVFPLAPSSKSTSGGTAALGCLVKDYFPEPVTVSWNSGALTSGVHTFPAVLQSSGLYSLSSVVTVPSSSLGTQTYICNVNHKPSNTKVDKRVEPKSCDKTHTCPPCPAPELLGGPSVFLFPPKPKDTLMISRTPEVTCVVVDVSHEDPEVKFNWYVDGVEVHNAKTKPREEQYNSTYRVVSVLTVLHQDWLNGKEYKCKVSNKALPAPIEKTISKAKGQPREPQVYTLPPSREEMTKNQVSLTCLVKGFYPSDIAVEWESNGQPENNYKTTPPVLDSDGSFFLYSKLTVDKSRWQQGNVFSCSVMHEALHNHYTQKSLSLSPGK